European Patent Application EP 4 703 390 A1, published March 4, 2026. Title: MULTISPECIFIC ANTIBODY TARGETING C-MET. Applicant: CHIA TAI TIANQING PHARMACEUTICAL GROUP CO., LTD. The sequence listing filed with the application follows.

SEQUENCE LISTING (92 sequences)

SEQ ID NO: 1 - skipped

SEQ ID NO: 2 - protein, 17 aa, synthetic construct
VINPGGDNTDYTYAVKG

SEQ ID NO: 3 - protein, 16 aa, synthetic construct
GRTFGGTWMDRNKWKY

SEQ ID NO: 4 - protein, 5 aa, synthetic construct
SGCMG

SEQ ID NO: 5 - protein, 17 aa, synthetic construct
  SITE 14: note = S or T
TIYTRNDFTYYSDXVKG

SEQ ID NO: 6 - protein, 22 aa, synthetic construct
GSPFRYAGAWNVCGLKEEDYNY

SEQ ID NO: 7 - protein, 5 aa, synthetic construct
ANCVG

SEQ ID NO: 8 - protein, 17 aa, synthetic construct
AINTGGETATYADFVKG

SEQ ID NO: 9 - protein, 19 aa, synthetic construct
VGTRKYWDECSLSQHAYKN

SEQ ID NO: 10 - protein, 5 aa, synthetic construct
SYAMD

SEQ ID NO: 11 - protein, 16 aa, synthetic construct
GINSAGSPSYEASVKG

SEQ ID NO: 12 - protein, 10 aa, synthetic construct
CRDFRSPYCR

SEQ ID NO: 13 - skipped

SEQ ID NO: 14 - protein, 16 aa, synthetic construct
SISSDGNSDYLDSVKG

SEQ ID NO: 15 - protein, 19 aa, synthetic construct
NGAGHLVLRPLCGSNAVDA

SEQ ID NO: 16 - protein, 5 aa, synthetic construct
GTTMG

SEQ ID NO: 17 - protein, 16 aa, synthetic construct
DISSDGNTYYSDSVKG

SEQ ID NO: 18 - protein, 18 aa, synthetic construct
AEFRLLLRPLCRQDDYGY

SEQ ID NO: 19 - protein, 5 aa, synthetic construct
YKYLA

SEQ ID NO: 20 - protein, 17 aa, synthetic construct
GLNTGGGSAYYADSVKG

SEQ ID NO: 21 - protein, 22 aa, synthetic construct
RRDYIHMTNIQALGLRPQWFSD

SEQ ID NO: 22 - protein, 5 aa, synthetic construct
SNFMA

SEQ ID NO: 23 - protein, 17 aa, synthetic construct
TITTGAGNTAYADSVKG

SEQ ID NO: 24 - protein, 13 aa, synthetic construct
GRGGFWRPAEYDF

SEQ ID NO: 25 - protein, 123 aa, synthetic construct
QVQLVESGGGSVQAGGSLRLSCVVSGYTYSSVAWFRQTPGKEREGVAVINPGGDNTDYTYAVKGRFTISRDSAKSTVFLQMNNLESEDTAMYYCAAGRTFGGTWMDRNKWKYWGQGTLVTVSS

SEQ ID NO: 26 - protein, 131 aa, synthetic construct
QVQLVESGGDSVQAGGSLRLSCAASAHAYSSGCMGWFRQAPGKGREGVATIYTRNDFTYYSDSVKGRFTISRDDAKNTVYLQVNSLKAEDTAMYYCAAGSPFRYAGAWNVCGLKEEDYNYWGQGTLVTVSS

SEQ ID NO: 27 - protein, 128 aa, synthetic construct
QVQLVESGGGLVQPGGSLRLSCAASGYSYSANCVGWFYQAPGKEREGVAAINTGGETATYADFVKGRFTISQDYAKNTVYLQMNSLKSEDTGMYYCAAVGTRKYWDECSLSQHAYKNWGQGTLVTVSS

SEQ ID NO: 28 - protein, 118 aa, synthetic construct
EVQLVESGGGLVQPGGSLRLSCVASGFTFKSYAMDWVRQAPGKGLEWIAGINSAGSPSYEASVKGRFTISRDNAENTLYLQLNSLKTEDTAMYYCTKCRDFRSPYCRPGQGTLVTVSS

SEQ ID NO: 29 - protein, 124 aa, synthetic construct
EVQLVESGGGSVQAGGSLRLSCTASGFTFDMGWYRQAPGDECELVSSISSDGNSDYLDSVKGRFTISQDNAKNTVYLQMNSLKPEDTAVYYCAANGAGHLVLRPLCGSNAVDAWGQGTLVTVSS

SEQ ID NO: 30 - protein, 126 aa, synthetic construct
QVQLVESGGDSVQAGGSLRLSCIASGFTFDGTTMGWYRQAPGDECELVSDISSDGNTYYSDSVKGRFTISQGNAKNTVYLQMNSLTPEDTAVYYCAAAEFRLLLRPLCRQDDYGYWGQGTLVTVSS

SEQ ID NO: 31 - protein, 131 aa, synthetic construct
QVQLQESGGGLVQPGGSLRLSCAASGTTGDYKYLAWFRQGPGKEREGIAGLNTGGGSAYYADSVKGRFTISQDNVKRLLYLQLNNLKPEDTAMYYCAARRDYIHMTNIQALGLRPQWFSDWGQGTQVTVSS

SEQ ID NO: 32 - protein, 122 aa, synthetic construct
EVQLVESGGGSVQAQGSLRLSCTVSGSTYSSNFMAWFRQAPGKEREWVATITTGAGNTAYADSVKGRFTISEDNAKRTAYLQMNSLKPEDTAVYYCAAGRGGFWRPAEYDFWGQGTQVTVSS

SEQ ID NO: 33 - protein, 131 aa, synthetic construct
QVQLLESGGGSVQAGGSLRLSCAASGFTFSSGCMGWFRQAPGKGREGVATIYTRNDFTYYSDSVKGRFTISRDNSKNTVYLQMNSLRAEDTAVYYCAAGSPFRYAGAWNVCGLKEEDYNYWGQGTLVTVSS

SEQ ID NO: 34 - protein, 131 aa, synthetic construct
QVQLLESGGGSVQAGGSLRLSCAASGHTYSSGCMGWFRQAPGKGREGVATIYTRNDFTYYSDSVKGRFTISRDNSKNTVYLQMNSLRAEDTAVYYCAAGSPFRYAGAWNVCGLKEEDYNYWGQGTLVTVSS

SEQ ID NO: 35 - protein, 131 aa, synthetic construct
QVQLLESGGGSVQAGGSLRLSCAASGHTYSSGCMGWFRQAPGKGREGVATIYTRNDFTYYSDTVKGRFTISRDNSKNTVYLQMNSLRAEDTAVYYCAAGSPFRYAGAWNVCGLKEEDYNYWGQGTLVTVSS

SEQ ID NO: 36 - protein, 128 aa, synthetic construct
QVQLVESGGGSVQPGGSLRLSCAASGYSYSANCVGWFRQAPGKGREGVSAINTGGETATYADFVKGRFTISRDNAKNTVYLQMNSLRAEDTAVYYCAAVGTRKYWDECSLSQHAYKNWGQGTLVTVSS

SEQ ID NO: 37 - protein, 128 aa, synthetic construct
QVQLVESGGGSVQPGGSLRLSCAASGFTFSANCVGWFRQAPGKGREGVSAINTGGETATYADFVKGRFTISRDNAKNTVYLQMNSLRAEDTAVYYCAAVGTRKYWDECSLSQHAYKNWGQGTLVTVSS

SEQ ID NO: 38 - protein, 122 aa, synthetic construct
EVQLVESGGGSVQAGGSLRLSCAVSGFTVSSNFMAWFRQAPGKGREWVSTITTGAGNTAYADSVKGRFTISEDNSKNTLYLQMNSLRAEDTAVYYCAAGRGGFWRPAEYDFWGQGTTVTVSS

SEQ ID NO: 39 - protein, 122 aa, synthetic construct
EVQLVESGGGSVQAGGSLRLSCAVSGFTVSSNFMAWFRQAPGKGREWVSTITTGAGNTAYADSVKGRFTISEDNSKNTAYLQMNSLRAEDTAVYYCAAGRGGFWRPAEYDFWGQGTTVTVSS

SEQ ID NO: 40 - protein, 131 aa, synthetic construct
  SITE 5: note = V or L
  SITE 10: note = D or G
  SITE 26: note = A or G
  SITE 27: note = H or F
  SITE 28: note = A or T
  SITE 29: note = Y or F
  SITE 63: note = S or T
  SITE 74: note = D or N
  SITE 75: note = A or S
  SITE 83: note = V or M
  SITE 87: note = K or R
  SITE 93: note = M or V
QVQLXESGGXSVQAGGSLRLSCAASXXXXSSGCMGWFRQAPGKGREGVATIYTRNDFTYYSDXVKGRFTISRDXXKNTVYLQXNSLXAEDTAXYYCAAGSPFRYAGAWNVCGLKEEDYNYWGQGTLVTVSS

SEQ ID NO: 41 - protein, 128 aa, synthetic construct
  SITE 11: note = L or S
  SITE 27: note = Y or F
  SITE 28: note = S or T
  SITE 29: note = Y or F
  SITE 38: note = Y or R
  SITE 44: note = E or G
  SITE 49: note = A or S
  SITE 72: note = Q or R
  SITE 74: note = Y or N
  SITE 87: note = K or R
  SITE 88: note = S or A
  SITE 92: note = G or A
  SITE 93: note = M or V
QVQLVESGGGXVQPGGSLRLSCAASGXXXSANCVGWFXQAPGKXREGVXAINTGGETATYADFVKGRFTISXDXAKNTVYLQMNSLXXEDTXXYYCAAVGTRKYWDECSLSQHAYKNWGQGTLVTVSS

SEQ ID NO: 42 - protein, 122 aa, synthetic construct
  SITE 15: note = Q or G
  SITE 23: note = T or A
  SITE 27: note = S or F
  SITE 29: note = Y or V
  SITE 44: note = E or G
  SITE 49: note = A or S
  SITE 75: note = A or S
  SITE 77: note = R or N
  SITE 79: note = A or L
  SITE 87: note = K or R
  SITE 88: note = P or A
  SITE 117: note = Q or T
EVQLVESGGGSVQAXGSLRLSCXVSGXTXSSNFMAWFRQAPGKXREWVXTITTGAGNTAYADSVKGRFTISEDNXKXTXYLQMNSLXXEDTAVYYCAAGRGGFWRPAEYDFWGQGTXVTVSS

SEQ ID NO: 43 - protein, 375 aa, synthetic construct
QVQLVESGGGSVQAGGSLRLSCVVSGYTYSSVAWFRQTPGKEREGVAVINPGGDNTDYTYAVKGRFTISRDSAKSTVFLQMNNLESEDTAMYYCAAGRTFGGTWMDRNKWKYWGQGTLVTVSSEPKIPQPQPKPQPQPQPQPKPQPKPEPECTCPKCPAPELLGGPSVFLFPPKPKDTLMISRTPEVTCVVVDVSHEDPEVKFNWYVDGVEVHNAKTKPREEQYNSTYRVVSVLTVLHQDWLNGKEYKCKVSNKALPAPIEKTISKAKGQPREPQVYTLPPSRDELTKNQVSLTCLVKGFYPSDIAVEWESNGQPENNYKTTPPVLDSDGSFFLYSKLTVDKSRWQQGNVFSCSVMHEALHNHYTQKSLSLSPGK

SEQ ID NO: 44 - protein, 383 aa, synthetic construct
QVQLVESGGDSVQAGGSLRLSCAASAHAYSSGCMGWFRQAPGKGREGVATIYTRNDFTYYSDSVKGRFTISRDDAKNTVYLQVNSLKAEDTAMYYCAAGSPFRYAGAWNVCGLKEEDYNYWGQGTLVTVSSEPKIPQPQPKPQPQPQPQPKPQPKPEPECTCPKCPAPELLGGPSVFLFPPKPKDTLMISRTPEVTCVVVDVSHEDPEVKFNWYVDGVEVHNAKTKPREEQYNSTYRVVSVLTVLHQDWLNGKEYKCKVSNKALPAPIEKTISKAKGQPREPQVYTLPPSRDELTKNQVSLTCLVKGFYPSDIAVEWESNGQPENNYKTTPPVLDSDGSFFLYSKLTVDKSRWQQGNVFSCSVMHEALHNHYTQKSLSLSPGK

SEQ ID NO: 45 - protein, 380 aa, synthetic construct
QVQLVESGGGLVQPGGSLRLSCAASGYSYSANCVGWFYQAPGKEREGVAAINTGGETATYADFVKGRFTISQDYAKNTVYLQMNSLKSEDTGMYYCAAVGTRKYWDECSLSQHAYKNWGQGTLVTVSSEPKIPQPQPKPQPQPQPQPKPQPKPEPECTCPKCPAPELLGGPSVFLFPPKPKDTLMISRTPEVTCVVVDVSHEDPEVKFNWYVDGVEVHNAKTKPREEQYNSTYRVVSVLTVLHQDWLNGKEYKCKVSNKALPAPIEKTISKAKGQPREPQVYTLPPSRDELTKNQVSLTCLVKGFYPSDIAVEWESNGQPENNYKTTPPVLDSDGSFFLYSKLTVDKSRWQQGNVFSCSVMHEALHNHYTQKSLSLSPGK

SEQ ID NO: 46 - protein, 370 aa, synthetic construct
EVQLVESGGGLVQPGGSLRLSCVASGFTFKSYAMDWVRQAPGKGLEWIAGINSAGSPSYEASVKGRFTISRDNAENTLYLQLNSLKTEDTAMYYCTKCRDFRSPYCRPGQGTLVTVSSEPKIPQPQPKPQPQPQPQPKPQPKPEPECTCPKCPAPELLGGPSVFLFPPKPKDTLMISRTPEVTCVVVDVSHEDPEVKFNWYVDGVEVHNAKTKPREEQYNSTYRVVSVLTVLHQDWLNGKEYKCKVSNKALPAPIEKTISKAKGQPREPQVYTLPPSRDELTKNQVSLTCLVKGFYPSDIAVEWESNGQPENNYKTTPPVLDSDGSFFLYSKLTVDKSRWQQGNVFSCSVMHEALHNHYTQKSLSLSPGK

SEQ ID NO: 47 - protein, 376 aa, synthetic construct
EVQLVESGGGSVQAGGSLRLSCTASGFTFDMGWYRQAPGDECELVSSISSDGNSDYLDSVKGRFTISQDNAKNTVYLQMNSLKPEDTAVYYCAANGAGHLVLRPLCGSNAVDAWGQGTLVTVSSEPKIPQPQPKPQPQPQPQPKPQPKPEPECTCPKCPAPELLGGPSVFLFPPKPKDTLMISRTPEVTCVVVDVSHEDPEVKFNWYVDGVEVHNAKTKPREEQYNSTYRVVSVLTVLHQDWLNGKEYKCKVSNKALPAPIEKTISKAKGQPREPQVYTLPPSRDELTKNQVSLTCLVKGFYPSDIAVEWESNGQPENNYKTTPPVLDSDGSFFLYSKLTVDKSRWQQGNVFSCSVMHEALHNHYTQKSLSLSPGK

SEQ ID NO: 48 - protein, 378 aa, synthetic construct
QVQLVESGGDSVQAGGSLRLSCIASGFTFDGTTMGWYRQAPGDECELVSDISSDGNTYYSDSVKGRFTISQGNAKNTVYLQMNSLTPEDTAVYYCAAAEFRLLLRPLCRQDDYGYWGQGTLVTVSSEPKIPQPQPKPQPQPQPQPKPQPKPEPECTCPKCPAPELLGGPSVFLFPPKPKDTLMISRTPEVTCVVVDVSHEDPEVKFNWYVDGVEVHNAKTKPREEQYNSTYRVVSVLTVLHQDWLNGKEYKCKVSNKALPAPIEKTISKAKGQPREPQVYTLPPSRDELTKNQVSLTCLVKGFYPSDIAVEWESNGQPENNYKTTPPVLDSDGSFFLYSKLTVDKSRWQQGNVFSCSVMHEALHNHYTQKSLSLSPGK

SEQ ID NO: 49 - protein, 363 aa, synthetic construct
QVQLQESGGGLVQPGGSLRLSCAASGTTGDYKYLAWFRQGPGKEREGIAGLNTGGGSAYYADSVKGRFTISQDNVKRLLYLQLNNLKPEDTAMYYCAARRDYIHMTNIQALGLRPQWFSDWGQGTQVTVSSEPKSSDKTHTCPPCPAPELLGGPSVFLFPPKPKDTLMISRTPEVTCVVVDVSHEDPEVKFNWYVDGVEVHNAKTKPREEQYNSTYRVVSVLTVLHQDWLNGKEYKCKVSNKALPAPIEKTISKAKGQPREPQVYTLPPSRDELTKNQVSLTCLVKGFYPSDIAVEWESNGQPENNYKTTPPVLDSDGSFFLYSKLTVDKSRWQQGNVFSCSVMHEALHNHYTQKSLSLSPGK

SEQ ID NO: 50 - protein, 354 aa, synthetic construct
EVQLVESGGGSVQAQGSLRLSCTVSGSTYSSNFMAWFRQAPGKEREWVATITTGAGNTAYADSVKGRFTISEDNAKRTAYLQMNSLKPEDTAVYYCAAGRGGFWRPAEYDFWGQGTQVTVSSEPKSSDKTHTCPPCPAPELLGGPSVFLFPPKPKDTLMISRTPEVTCVVVDVSHEDPEVKFNWYVDGVEVHNAKTKPREEQYNSTYRVVSVLTVLHQDWLNGKEYKCKVSNKALPAPIEKTISKAKGQPREPQVYTLPPSRDELTKNQVSLTCLVKGFYPSDIAVEWESNGQPENNYKTTPPVLDSDGSFFLYSKLTVDKSRWQQGNVFSCSVMHEALHNHYTQKSLSLSPGK

SEQ ID NO: 51 - protein, 364 aa, synthetic construct
QVQLLESGGGSVQAGGSLRLSCAASGFTFSSGCMGWFRQAPGKGREGVATIYTRNDFTYYSDSVKGRFTISRDNSKNTVYLQMNSLRAEDTAVYYCAAGSPFRYAGAWNVCGLKEEDYNYWGQGTLVTVSSGEPKSSDKTHTCPPCPAPELLGGPSVFLFPPKPKDTLMISRTPEVTCVVVDVSHEDPEVKFNWYVDGVEVHNAKTKPREEQYNSTYRVVSVLTVLHQDWLNGKEYKCKVSNKALPAPIEKTISKAKGQPREPQVYTLPPSRDELTKNQVSLTCLVKGFYPSDIAVEWESNGQPENNYKTTPPVLDSDGSFFLYSKLTVDKSRWQQGNVFSCSVMHEALHNHYTQKSLSLSPGK

SEQ ID NO: 52 - DNA, 1092 bp, synthetic construct
  source 1..1092: mol_type = other DNA
caggtgcagctgctggagagcggcggcggaagcgtgcaggctggaggatccctgcggctgagctgtgctgcctccggcttcaccttcagctccggctgcatgggctggttcaggcaggcccctggcaagggccgggagggagttgctaccatctacacccggaatgacttcacctattactccgacagcgtgaagggcaggttcaccatcagccgggacaactccaagaacaccgtgtatctgcagatgaatagcctgcgggccgaggacaccgccgtgtactattgcgctgccggcagccccttcaggtacgctggcgcttggaatgtgtgtggcctgaaggaggaggattacaattattggggccagggcaccctggtgaccgtgagcagcggagagccaaagtccagcgataagacccacacctgccccccttgccctgctcccgagctgctgggaggccctagcgtgttcctgttcccccctaagcctaaggacaccctgatgatcagccggacccccgaggtgacctgtgtggtggtggatgtgagccacgaggatcctgaggtgaagttcaactggtatgtggacggcgtggaggtgcacaacgccaagaccaagcctagggaggagcagtataactccacctatagggtggtgagcgtgctgaccgtgctgcaccaggattggctgaatggcaaggagtacaagtgcaaggtgagcaataaggctctgcctgctcctatcgagaagaccatctccaaggctaagggccagcccagggagcctcaggtgtacaccctgcctcccagcagggacgagctgaccaagaatcaggtgagcctgacctgcctggtgaagggcttctacccctccgatatcgctgtggagtgggagagcaacggccagcctgagaacaactacaagaccaccccccccgtgctggattccgatggctccttcttcctgtacagcaagctgaccgtggataagagccggtggcagcagggcaacgtgttcagctgctccgtgatgcacgaggccctgcacaaccactacacccagaagagcctgagcctgagccctggcaag

SEQ ID NO: 53 - protein, 364 aa, synthetic construct
QVQLLESGGGSVQAGGSLRLSCAASGHTYSSGCMGWFRQAPGKGREGVATIYTRNDFTYYSDSVKGRFTISRDNSKNTVYLQMNSLRAEDTAVYYCAAGSPFRYAGAWNVCGLKEEDYNYWGQGTLVTVSSGEPKSSDKTHTCPPCPAPELLGGPSVFLFPPKPKDTLMISRTPEVTCVVVDVSHEDPEVKFNWYVDGVEVHNAKTKPREEQYNSTYRVVSVLTVLHQDWLNGKEYKCKVSNKALPAPIEKTISKAKGQPREPQVYTLPPSRDELTKNQVSLTCLVKGFYPSDIAVEWESNGQPENNYKTTPPVLDSDGSFFLYSKLTVDKSRWQQGNVFSCSVMHEALHNHYTQKSLSLSPGK

SEQ ID NO: 54 - DNA, 1092 bp, synthetic construct
  source 1..1092: mol_type = other DNA
caggtgcagctgctggagtccggcggcggatccgtgcaggctggaggatccctgcggctgagctgcgctgcttccggccacacctactcctccggctgcatgggctggttcaggcaggctcctggcaagggccgggagggagtggctaccatctataccaggaacgacttcacctactattccgattccgtgaagggcaggttcaccatcagcagggataactccaagaacaccgtgtatctgcagatgaatagcctgcgggccgaggataccgccgtgtactactgcgccgccggcagccccttccggtacgctggagcttggaacgtgtgcggcctgaaggaggaggactacaactattggggccagggcaccctggtgaccgtgagctccggagagccaaagtccagcgataagacccacacctgccccccttgccctgctcccgagctgctgggaggccctagcgtgttcctgttcccccctaagcctaaggacaccctgatgatcagccggacccccgaggtgacctgtgtggtggtggatgtgagccacgaggatcctgaggtgaagttcaactggtatgtggacggcgtggaggtgcacaacgccaagaccaagcctagggaggagcagtataactccacctatagggtggtgagcgtgctgaccgtgctgcaccaggattggctgaatggcaaggagtacaagtgcaaggtgagcaataaggctctgcctgctcctatcgagaagaccatctccaaggctaagggccagcccagggagcctcaggtgtacaccctgcctcccagcagggacgagctgaccaagaatcaggtgagcctgacctgcctggtgaagggcttctacccctccgatatcgctgtggagtgggagagcaacggccagcctgagaacaactacaagaccaccccccccgtgctggattccgatggctccttcttcctgtacagcaagctgaccgtggataagagccggtggcagcagggcaacgtgttcagctgctccgtgatgcacgaggccctgcacaaccactacacccagaagagcctgagcctgagccctggcaag

SEQ ID NO: 55 - protein, 364 aa, synthetic construct
QVQLLESGGGSVQAGGSLRLSCAASGHTYSSGCMGWFRQAPGKGREGVATIYTRNDFTYYSDTVKGRFTISRDNSKNTVYLQMNSLRAEDTAVYYCAAGSPFRYAGAWNVCGLKEEDYNYWGQGTLVTVSSGEPKSSDKTHTCPPCPAPELLGGPSVFLFPPKPKDTLMISRTPEVTCVVVDVSHEDPEVKFNWYVDGVEVHNAKTKPREEQYNSTYRVVSVLTVLHQDWLNGKEYKCKVSNKALPAPIEKTISKAKGQPREPQVYTLPPSRDELTKNQVSLTCLVKGFYPSDIAVEWESNGQPENNYKTTPPVLDSDGSFFLYSKLTVDKSRWQQGNVFSCSVMHEALHNHYTQKSLSLSPGK

SEQ ID NO: 56 - DNA, 1092 bp, synthetic construct
  source 1..1092: mol_type = other DNA
caggtgcagctgctggagagcggcggcggaagcgtgcaggctggaggaagcctgaggctgagctgcgccgccagcggacacacctacagctccggctgtatgggctggttcaggcaggcccccggcaagggacgggagggagttgctaccatctacacccggaatgacttcacctactattccgataccgtgaagggcaggttcaccatcagcagggacaactccaagaataccgtgtacctgcagatgaactccctgcgggccgaggacaccgccgtgtattactgtgctgctggctcccccttcaggtatgccggcgcttggaatgtgtgcggcctgaaggaggaggactataattattggggccagggcaccctggtgaccgtgagcagcggagagccaaagtccagcgataagacccacacctgccccccttgccctgctcccgagctgctgggaggccctagcgtgttcctgttcccccctaagcctaaggacaccctgatgatcagccggacccccgaggtgacctgtgtggtggtggatgtgagccacgaggatcctgaggtgaagttcaactggtatgtggacggcgtggaggtgcacaacgccaagaccaagcctagggaggagcagtataactccacctatagggtggtgagcgtgctgaccgtgctgcaccaggattggctgaatggcaaggagtacaagtgcaaggtgagcaataaggctctgcctgctcctatcgagaagaccatctccaaggctaagggccagcccagggagcctcaggtgtacaccctgcctcccagcagggacgagctgaccaagaatcaggtgagcctgacctgcctggtgaagggcttctacccctccgatatcgctgtggagtgggagagcaacggccagcctgagaacaactacaagaccaccccccccgtgctggattccgatggctccttcttcctgtacagcaagctgaccgtggataagagccggtggcagcagggcaacgtgttcagctgctccgtgatgcacgaggccctgcacaaccactacacccagaagagcctgagcctgagccctggcaag

SEQ ID NO: 57 - protein, 361 aa, synthetic construct
QVQLVESGGGSVQPGGSLRLSCAASGYSYSANCVGWFRQAPGKGREGVSAINTGGETATYADFVKGRFTISRDNAKNTVYLQMNSLRAEDTAVYYCAAVGTRKYWDECSLSQHAYKNWGQGTLVTVSSGEPKSSDKTHTCPPCPAPELLGGPSVFLFPPKPKDTLMISRTPEVTCVVVDVSHEDPEVKFNWYVDGVEVHNAKTKPREEQYNSTYRVVSVLTVLHQDWLNGKEYKCKVSNKALPAPIEKTISKAKGQPREPQVYTLPPSRDELTKNQVSLTCLVKGFYPSDIAVEWESNGQPENNYKTTPPVLDSDGSFFLYSKLTVDKSRWQQGNVFSCSVMHEALHNHYTQKSLSLSPGK

SEQ ID NO: 58 - DNA, 1083 bp, synthetic construct
  source 1..1083: mol_type = other DNA
caggtgcagctggtggagtccggcggcggaagcgtgcagcctggaggaagcctgaggctgtcctgcgctgcctccggctatagctacagcgctaactgcgtgggctggttccggcaggctcctggcaagggccgggagggagtgtccgctatcaacaccggcggcgagaccgctacctacgccgacttcgtgaagggccggttcaccatctcccgggataacgctaagaataccgtgtacctgcagatgaatagcctgcgggctgaggataccgccgtgtattattgtgctgccgtgggcacccggaagtactgggacgagtgcagcctgagccagcacgcctacaagaattggggccagggcaccctggtgaccgtgtccagcggagagccaaagtccagcgataagacccacacctgccccccttgccctgctcccgagctgctgggaggccctagcgtgttcctgttcccccctaagcctaaggacaccctgatgatcagccggacccccgaggtgacctgtgtggtggtggatgtgagccacgaggatcctgaggtgaagttcaactggtatgtggacggcgtggaggtgcacaacgccaagaccaagcctagggaggagcagtataactccacctatagggtggtgagcgtgctgaccgtgctgcaccaggattggctgaatggcaaggagtacaagtgcaaggtgagcaataaggctctgcctgctcctatcgagaagaccatctccaaggctaagggccagcccagggagcctcaggtgtacaccctgcctcccagcagggacgagctgaccaagaatcaggtgagcctgacctgcctggtgaagggcttctacccctccgatatcgctgtggagtgggagagcaacggccagcctgagaacaactacaagaccaccccccccgtgctggattccgatggctccttcttcctgtacagcaagctgaccgtggataagagccggtggcagcagggcaacgtgttcagctgctccgtgatgcacgaggccctgcacaaccactacacccagaagagcctgagcctgagccctggcaag

SEQ ID NO: 59 - protein, 361 aa, synthetic construct
QVQLVESGGGSVQPGGSLRLSCAASGFTFSANCVGWFRQAPGKGREGVSAINTGGETATYADFVKGRFTISRDNAKNTVYLQMNSLRAEDTAVYYCAAVGTRKYWDECSLSQHAYKNWGQGTLVTVSSGEPKSSDKTHTCPPCPAPELLGGPSVFLFPPKPKDTLMISRTPEVTCVVVDVSHEDPEVKFNWYVDGVEVHNAKTKPREEQYNSTYRVVSVLTVLHQDWLNGKEYKCKVSNKALPAPIEKTISKAKGQPREPQVYTLPPSRDELTKNQVSLTCLVKGFYPSDIAVEWESNGQPENNYKTTPPVLDSDGSFFLYSKLTVDKSRWQQGNVFSCSVMHEALHNHYTQKSLSLSPGK

SEQ ID NO: 60 - DNA, 1083 bp, synthetic construct
  source 1..1083: mol_type = other DNA
caggtgcagctggtggagtccggcggcggatccgtgcagcctggaggatccctgaggctgagctgcgccgccagcggattcaccttcagcgccaactgcgtgggctggttccggcaggctcctggcaagggccgggagggagtgagcgctatcaacaccggcggcgagaccgccacctatgccgacttcgtgaagggccggttcaccatctccagggataatgctaagaacaccgtgtacctgcagatgaatagcctgagggccgaggataccgccgtgtattactgtgccgccgtgggcaccaggaagtattgggacgagtgctccctgtcccagcacgcttacaagaactggggccagggcaccctggtgaccgtgagcagcggagagccaaagtccagcgataagacccacacctgccccccttgccctgctcccgagctgctgggaggccctagcgtgttcctgttcccccctaagcctaaggacaccctgatgatcagccggacccccgaggtgacctgtgtggtggtggatgtgagccacgaggatcctgaggtgaagttcaactggtatgtggacggcgtggaggtgcacaacgccaagaccaagcctagggaggagcagtataactccacctatagggtggtgagcgtgctgaccgtgctgcaccaggattggctgaatggcaaggagtacaagtgcaaggtgagcaataaggctctgcctgctcctatcgagaagaccatctccaaggctaagggccagcccagggagcctcaggtgtacaccctgcctcccagcagggacgagctgaccaagaatcaggtgagcctgacctgcctggtgaagggcttctacccctccgatatcgctgtggagtgggagagcaacggccagcctgagaacaactacaagaccaccccccccgtgctggattccgatggctccttcttcctgtacagcaagctgaccgtggataagagccggtggcagcagggcaacgtgttcagctgctccgtgatgcacgaggccctgcacaaccactacacccagaagagcctgagcctgagccctggcaag

SEQ ID NO: 61 - protein, 463 aa, synthetic construct
QRKRRNTIHEFKKSAKTTLIKIDPALKIKTKKVNTADQCANRCTRNKGLPFTCKAFVFDKARKQCLWFPFNSMSSGVKKEFGHEFDLYENKDYIRNCIIGKGRSYKGTVSITKSGIKCQPWSSMIPHEHSFLPSSYRGKDLQENYCRNPRGEEGGPWCFTSNPEVRYEVCDIPQCSEVECMTCNGESYRGLMDHTESGKICQRWDHQTPHRHKFLPERYPDKGFDDNYCRNPDGQPRPWCYTLDPHTRWEYCAIKTCADNTMNDTDVPLETTECIQGQGEGYRGTVNTIWNGIPCQRWDSQYPHEHDMTPENFKCKDLRENYCRNPDGSESPWCFTTDPNIRVGYCSQIPNCDMSHGQDCYRGNGKNYMGNLSQTRSGLTCSMWDKNMEDLHRHIFWEPDASKLNENYCRNPDDDAHGPWCYTGNPLIPWDYCPISRCEGDTTPTIVNLDHPVISCAKTKQLR

SEQ ID NO: 62 - protein, 234 aa, synthetic construct
VVNGIPTRTNIGWMVSLRYRNKHICGGSLIKESWVLTARQCFPSRDLKDYEAWLGIHDVHGRGDEKCKQVLNVSQLVYGPEGSDLVLMKLARPAVLDDFVSTIDLPNYGCTIPEKTSCSVYGWGYTGLINYDGLLRVAHLYIMGNEKCSQHHRGKVTLNESEICAGAEKIGSGPCEGDYGGPLVCEQHKMRMVLGVIVPGRGCAIPNRPGIFVRVAYYAKWIHKIILTYKVPQS

SEQ ID NO: 63 - protein, 5 aa, synthetic construct
TYGMH

SEQ ID NO: 64 - protein, 17 aa, synthetic construct
VIWDDGSYKYYGDSVKG

SEQ ID NO: 65 - protein, 16 aa, synthetic construct
DGITMVRGVMKDYFDY

SEQ ID NO: 66 - protein, 11 aa, synthetic construct
RASQDISSALV

SEQ ID NO: 67 - protein, 7 aa, synthetic construct
DASSLES

SEQ ID NO: 68 - protein, 9 aa, synthetic construct
QQFNSYPLT

SEQ ID NO: 69 - protein, 125 aa, synthetic construct [sequence omitted]

SEQ ID NO: 70 - protein, 107 aa, synthetic construct [sequence omitted]

SEQ ID NO: 71 - protein, 502 aa, synthetic construct
QVQLVESGGDSVQAGGSLRLSCAASAHAYSSGCMGWFRQAPGKGREGVATIYTRNDFTYYSDSVKGRFTISRDDAKNTVYLQVNSLKAEDTAMYYCAAGSPFRYAGAWNVCGLKEEDYNYWGQGTLVTVSSGGGGSGGGGSQVQLVESGGGLVQPGGSLRLSCAASGYSYSANCVGWFYQAPGKEREGVAAINTGGETATYADFVKGRFTISQDYAKNTVYLQMNSLKSEDTGMYYCAAVGTRKYWDECSLSQHAYKNWGQGTLVTVSSGEPKSSDKTHTCPPCPAPELLGGPSVFLFPPKPKDTLMISRTPEVTCVVVDVSHEDPEVKFNWYVDGVEVHNAKTKPREEQYNSTYRVVSVLTVLHQDWLNGKEYKCKVSNKALPAPIEKTISKAKGQPREPQVCTLPPSREEMTKNQVSLSCAVKGFYPSDIAVEWESNGQPENNYKTTPPVLDSDGSFFLVSKLTVDKSRWQQGNVFSCSVMHEALHNRFTQKSLSLSPGK

SEQ ID NO: 72 - DNA, 1506 bp, synthetic construct
  source 1..1506: mol_type = other DNA
caagtgcagctggtcgagtccggcggcgactccgtgcaggctggcggatctctgagactgtcttgcgctgcttctgcccacgcttactccagcggctgcatgggctggttcagacaggcccctggcaagggcagagaaggagtggctaccatctacaccagaaacgactttacctattactccgattctgtcaagggcaggttcaccatctcccgggacgacgccaagaacaccgtgtacctgcaggtgaacagcctgaaggccgaggataccgccatgtactactgcgccgctggctcccctttccggtatgccggcgcctggaacgtgtgcggcctgaaagaagaagactacaactactggggccagggaaccttggtgaccgtctcatccgggggcggcggtagcggtggcggaggctctcaagtgcagctggtggaatctggcggaggactggttcagcctggcggctctctccggctgtcctgcgccgcctctggctactcctactctgccaactgcgtgggctggttctaccaggcccccggcaaggagagagagggcgtggccgccatcaacaccggcggcgagacagcaacctacgccgacttcgtgaaaggccggtttacaatctctcaggattatgctaagaataccgtgtacctgcagatgaactccctgaagtccgaggacacaggcatgtactactgtgctgctgtgggcacccggaagtactgggacgagtgctctctgagccagcacgcctacaaaaattggggccaaggcaccctggtgaccgtgtccagtggcgaacccaagtcctccgacaagacccacacctgccccccctgtcctgctccagagctgctgggcggcccttctgtgtttctgttccctcctaagcccaaggacaccctgatgatctccagaacccctgaggtgacctgtgtggtggtggacgtgtctcacgaggatcctgaagtgaagttcaactggtacgtggacggcgtggaagtgcataacgccaagacaaagcctagagaggaacagtacaactctacctacagagtggtgtccgtgctgaccgtgctgcaccaggactggctgaacggcaaagagtacaagtgcaaggtgtccaacaaggctctgcctgcccctatcgagaagaccatcagcaaggccaagggccagccccgcgagcctcaggtctgcaccctgcctccatccagagaagagatgaccaagaaccaggtttccctgtcttgtgctgtgaagggcttctaccctagcgacatcgccgtggaatgggagtctaatggccagcctgagaacaactacaagaccacacctcctgtgctcgactccgatggctccttcttcctggtgtccaagctgacggtggataagtctagatggcagcagggcaacgtgttctcctgctccgtgatgcacgaggccctgcataaccggttcacccagaagagcctgtccctgtctccaggaaaa

SEQ ID NO: 73 - protein, 502 aa, synthetic construct
QVQLLESGGGSVQAGGSLRLSCAASGFTFSSGCMGWFRQAPGKGREGVATIYTRNDFTYYSDSVKGRFTISRDNSKNTVYLQMNSLRAEDTAVYYCAAGSPFRYAGAWNVCGLKEEDYNYWGQGTLVTVSSGGGGSGGGGSQVQLVESGGGSVQPGGSLRLSCAASGYSYSANCVGWFRQAPGKGREGVSAINTGGETATYADFVKGRFTISRDNAKNTVYLQMNSLRAEDTAVYYCAAVGTRKYWDECSLSQHAYKNWGQGTLVTVSSGEPKSSDKTHTCPPCPAPELLGGPSVFLFPPKPKDTLMISRTPEVTCVVVDVSHEDPEVKFNWYVDGVEVHNAKTKPREEQYNSTYRVVSVLTVLHQDWLNGKEYKCKVSNKALPAPIEKTISKAKGQPREPQVCTLPPSREEMTKNQVSLSCAVKGFYPSDIAVEWESNGQPENNYKTTPPVLDSDGSFFLVSKLTVDKSRWQQGNVFSCSVMHEALHNRFTQKSLSLSPGK

SEQ ID NO: 74 - DNA, 1506 bp, synthetic construct
  source 1..1506: mol_type = other DNA
caggtgcagctgctggaatctggcggcggctctgtgcaggctggtggatccctgagactgtcttgtgctgcctccggctttaccttcagcagtggctgcatgggctggtttagacaggcccccggcaaaggcagagaaggcgtggccaccatctacaccagaaacgacttcacctattattccgattccgtgaaaggcagattcaccatcagccgcgacaactccaaaaacaccgtgtacctgcagatgaactccctgagagccgaggataccgctgtgtactactgcgccgccggctctcctttccggtacgccggagcttggaacgtgtgtggcctgaaggaagaggactacaactactggggacaaggcaccctggtgaccgtgtctagcggcggaggtggctcgggcggaggcggctctcaagtgcagctggtggaatccggcggcggctccgtgcaacccggaggctccctgcggttgtcctgtgctgcctctggctactcctactccgccaactgcgtaggatggttcagacaggcccctggcaagggcagagagggcgtgtccgctatcaacaccggcggcgagacagccacctacgccgacttcgtgaagggccggttcaccatctctcgggacaacgccaagaacactgtctatctgcagatgaactccctgagagcagaagataccgccgtgtactactgtgctgctgtgggcacccggaagtactgggacgagtgctctctgtcccagcacgcctacaagaattggggccagggcacactagtcaccgtctcctctggcgagcctaagtcctctgataagacccacacctgtcctccttgccctgctcctgagctgctgggcggcccttccgtcttcctgttccctccaaagcccaaggacacactgatgatctccaggacacctgaagtgacctgcgtggtggtggacgtgtctcatgaggaccccgaggtgaagttcaactggtacgtggatggcgtggaagtgcacaatgccaagaccaagcctcgggaggaacagtacaactctacctacagagtggtgtccgtgctgaccgtcctgcaccaggactggctgaacggcaaagagtacaagtgcaaggtgtccaacaaggccctgccagctcctatcgagaagacaatcagcaaggccaagggccagcctagagagcctcaggtgtgcaccctgcctccttctcgggaagagatgaccaagaaccaggtgagcctgtcctgcgccgtgaaaggcttctacccctccgacatcgccgtcgagtgggagtctaatggacagcccgagaacaactacaagaccacccctcctgtgctggactccgacggctctttcttcctggtttctaagctgaccgtggacaagtccagatggcagcagggcaacgtgttctcctgctccgtgatgcacgaagctctgcacaaccggtttacccagaagtctctgtctctcagcccaggcaag

SEQ ID NO: 75 - protein, 502 aa, synthetic construct
QVQLLESGGGSVQAGGSLRLSCAASGHTYSSGCMGWFRQAPGKGREGVATIYTRNDFTYYSDSVKGRFTISRDNSKNTVYLQMNSLRAEDTAVYYCAAGSPFRYAGAWNVCGLKEEDYNYWGQGTLVTVSSGGGGSGGGGSQVQLVESGGGSVQPGGSLRLSCAASGYSYSANCVGWFRQAPGKGREGVSAINTGGETATYADFVKGRFTISRDNAKNTVYLQMNSLRAEDTAVYYCAAVGTRKYWDECSLSQHAYKNWGQGTLVTVSSGEPKSSDKTHTCPPCPAPELLGGPSVFLFPPKPKDTLMISRTPEVTCVVVDVSHEDPEVKFNWYVDGVEVHNAKTKPREEQYNSTYRVVSVLTVLHQDWLNGKEYKCKVSNKALPAPIEKTISKAKGQPREPQVCTLPPSREEMTKNQVSLSCAVKGFYPSDIAVEWESNGQPENNYKTTPPVLDSDGSFFLVSKLTVDKSRWQQGNVFSCSVMHEALHNRFTQKSLSLSPGK

SEQ ID NO: 76 - DNA, 1506 bp, synthetic construct
  source 1..1506: mol_type = other DNA
caggttcagctgttggaatctggcggcggatctgttcaggctggcggatctctgagactgtcttgtgctgcttccggccacacctactcctctggctgtatgggatggttcagacaggcccctggcaagggaagagaaggcgtggccaccatctacacccggaacgacttcacctactactccgactccgtgaagggcagattcaccatcagccgggacaactccaagaacaccgtgtacctgcagatgaactccctgagagccgaggacaccgccgtgtactattgtgccgctggcagcccctttagatacgctggcgcttggaacgtgtgcggcctgaaagaagaggactacaactactggggccagggcaccctggtcacagtttctagcggaggcggaggatcaggtggcggtggatctcaggtgcagttggttgaaagtggcggaggctctgtgcaaccaggcggaagcctcagattgtcttgcgccgcttctggctactcctacagcgccaattgtgtcggctggtttaggcaggctcccggaaaaggcagagaaggggtgtccgctatcaacaccggcggagagacagccacctacgccgatttcgtgaaaggccggtttaccatctctcgcgataacgctaagaacacagtctatctccaaatgaacagcctgcgcgctgaggataccgctgtgtattactgcgctgccgtgggcaccagaaagtactgggacgagtgctccctgagccagcacgcctataagaattggggacagggaaccctcgtgaccgtgtcctctggcgaacctaagtcctccgacaagacccacacctgtcctccatgtcctgctccagaactgctcggcggaccttccgtgttcctgtttcctccaaagcctaaggacaccctgatgatctctcggacccctgaagtgacctgcgtggtggtggatgtgtctcacgaggatcccgaagtgaagttcaattggtacgtggacggcgtggaagtgcacaacgccaagaccaagcctagagaggaacagtacaactccacctacagagtggtgtccgtgctgaccgtgctgcaccaggattggctgaacggcaaagagtacaagtgcaaggtgtccaacaaggccctgcctgctcctatcgaaaagaccatctccaaggccaagggccagcctcgggaacctcaagtctgtaccctgcctcctagccgggaagagatgaccaagaaccaggtgtccctgtcctgcgctgtgaagggcttctacccttccgatatcgccgtggaatgggagagcaatggccagccagagaacaactacaagacaacccctcctgtgctggactccgacggctcattcttcctggtgtccaagctgacagtggacaagtccagatggcagcagggcaacgtgttctcctgctccgtgatgcacgaggccctgcacaacaggttcacccagaagtccctgtctctgagcccaggcaaa

SEQ ID NO: 77 - protein, 502 aa, synthetic construct
QVQLLESGGGSVQAGGSLRLSCAASGHTYSSGCMGWFRQAPGKGREGVATIYTRNDFTYYSDTVKGRFTISRDNSKNTVYLQMNSLRAEDTAVYYCAAGSPFRYAGAWNVCGLKEEDYNYWGQGTLVTVSSGGGGSGGGGSQVQLVESGGGSVQPGGSLRLSCAASGYSYSANCVGWFRQAPGKGREGVSAINTGGETATYADFVKGRFTISRDNAKNTVYLQMNSLRAEDTAVYYCAAVGTRKYWDECSLSQHAYKNWGQGTLVTVSSGEPKSSDKTHTCPPCPAPELLGGPSVFLFPPKPKDTLMISRTPEVTCVVVDVSHEDPEVKFNWYVDGVEVHNAKTKPREEQYNSTYRVVSVLTVLHQDWLNGKEYKCKVSNKALPAPIEKTISKAKGQPREPQVCTLPPSREEMTKNQVSLSCAVKGFYPSDIAVEWESNGQPENNYKTTPPVLDSDGSFFLVSKLTVDKSRWQQGNVFSCSVMHEALHNRFTQKSLSLSPGK

SEQ ID NO: 78 - DNA, 1506 bp, synthetic construct
  source 1..1506: mol_type = other DNA
caggttcagctgctggaatctggcggaggctccgtgcaggccggcggaagcctgagactgtcctgcgccgcctctggccatacatattcttccggctgcatgggctggttccggcaggctcctggcaagggcagggagggcgtggccacaatctacaccagaaacgacttcacctattattctgataccgtcaaaggcagattcaccatctctcgggacaactccaagaacaccgtgtacctgcagatgaactccctgcgggctgaggacaccgccgtctactactgcgccgctggctctccttttagatacgctggcgcctggaacgtgtgtggcctgaaggaagaagactacaactactggggccaaggcaccctggtgaccgtgtcctccggcggcggaggctctggaggcggcggcagccaagtgcagctggtggaaagcggcggtggctccgtgcagccaggcggctctctgcggctgtcctgtgccgcttctggctactcctactccgccaactgcgtgggctggttcagacaggcccccggcaagggccgggaaggcgtgtctgccatcaacaccggcggcgagacagctacctacgccgacttcgtgaagggcagatttaccatctccagagataacgctaagaataccgtgtacctgcagatgaacagcctgcgggccgaggacaccgctgtgtactactgtgctgccgtgggcacccggaagtactgggacgagtgcagtctgagccagcacgcctacaagaattggggccagggaacactggtcaccgtgtccagtggagaacctaagtcgtctgacaagacccacacctgtcctccatgccccgctcccgagctgctgggcggcccttctgtgttcctgttccctcctaagcccaaggacacactgatgatcagcagaacccctgaagtgacctgcgtggtggtggacgtgtcccacgaggatcctgaggtgaagttcaactggtacgtggacggcgtggaagtgcacaacgccaagaccaagcctcgcgaggagcagtacaactccacctacagagtggtctctgtactgaccgtgctgcaccaggactggctgaacggaaaagagtacaagtgcaaggtgtccaacaaggctctgcctgcccctatcgagaagaccatctccaaggccaaaggacagcctagagagcctcaagtgtgcaccctgcctccatctcgggaagagatgactaagaaccaggtctccctgtcctgtgccgtcaagggcttctacccctccgacatcgccgtggagtgggagtccaacggccagcctgagaacaactacaaaaccacacctcctgtgctggacagcgatggctccttcttcctcgtgtccaagctgaccgttgataagtccagatggcagcagggcaacgtgttctcttgctccgtgatgcacgaggccctgcataatagatttacccagaagtctctgtcgctctctcccggcaaa

SEQ ID NO: 79 - protein, 488 aa, synthetic construct
EVQLVESGGGSVQAQGSLRLSCTVSGSTYSSNFMAWFRQAPGKEREWVATITTGAGNTAYADSVKGRFTISEDNAKRTAYLQMNSLKPEDTAVYYCAAGRGGFWRPAEYDFWGQGTQVTVSSGGGGSQVQLVESGGGSVQPGGSLRLSCAASGYSYSANCVGWFRQAPGKGREGVSAINTGGETATYADFVKGRFTISRDNAKNTVYLQMNSLRAEDTAVYYCAAVGTRKYWDECSLSQHAYKNWGQGTLVTVSSGEPKSSDKTHTCPPCPAPELLGGPSVFLFPPKPKDTLMISRTPEVTCVVVDVSHEDPEVKFNWYVDGVEVHNAKTKPREEQYNSTYRVVSVLTVLHQDWLNGKEYKCKVSNKALPAPIEKTISKAKGQPREPQVCTLPPSREEMTKNQVSLSCAVKGFYPSDIAVEWESNGQPENNYKTTPPVLDSDGSFFLVSKLTVDKSRWQQGNVFSCSVMHEALHNRYTQKSLSLSPGK

SEQ ID NO: 80 - DNA, 1464 bp, synthetic construct
  source 1..1464: mol_type = other DNA
gaagtgcagctggtcgagtctggcggcggctctgtgcaggctcagggctccctgcggctgtcttgtaccgtttccgggtccacctactcttccaacttcatggcctggttccggcaggcccctggaaaagagagagaatgggtggctaccatcaccacaggcgctggcaacaccgcttatgccgactccgtcaagggcagattcaccatctctgaggacaacgccaagcggaccgcctacctgcagatgaacagcctgaagcctgaagataccgccgtgtactactgtgctgccggcagaggcggcttttggcggcccgctgagtacgacttctggggccaaggcactcaagtgacagtgtcctctggaggaggaggctctcaggtgcagctggtggaatctggcggcggctccgtgcaaccaggcggatctctgagactgtcctgcgctgcttccggctactcctactccgccaactgcgtgggctggttcagacaggcccctggcaaaggccgcgagggcgtctctgccatcaacaccggcggagagacagctacctacgccgattttgttaagggccggttcactatctccagagacaatgctaagaacaccgtgtacctgcagatgaactctctgagagccgaggacaccgctgtgtactactgcgccgctgtgggcacccggaagtactgggacgagtgctctctgtcccagcacgcctataagaattggggccagggcaccctcgtgaccgtgtcttcaggcgagcctaaaagcagcgataagacccacacctgccctccttgccccgctcctgagctgctgggcggaccttctgtctttctgttcccacctaagcccaaggacaccctgatgatcagccggacacctgaggtgacctgtgtggtggtggacgtgtctcatgaggatcctgaggtgaagttcaactggtacgtggatggcgtggaagtgcacaatgccaagaccaagcctagagaagagcagtacaactccacatacagagtggtctcggtgctgaccgtgctgcaccaggactggctgaacggcaaagaatacaagtgcaaggtgtccaacaaggctctgcctgcccccatcgagaagacaatctccaaggccaagggccagcctcgggaacctcaggtgtgcaccctgcccccctccagggaagaaatgacaaagaaccaggtgtccctatcctgtgccgtgaaaggcttctacccttccgacatcgccgtggagtgggagtccaacggccagcccgagaacaactacaaaaccacccctccagtgctggactctgacggctccttcttcctggtgagcaagctgaccgtggacaagtctagatggcaacagggaaacgtgttcagctgctccgtcatgcacgaggccctgcacaacagatacacccagaagtccctgagcctgtctcctggcaag

SEQ ID NO: 81 - protein, 488 aa, synthetic construct
EVQLVESGGGSVQAGGSLRLSCAVSGFTVSSNFMAWFRQAPGKGREWVSTITTGAGNTAYADSVKGRFTISEDNSKNTLYLQMNSLRAEDTAVYYCAAGRGGFWRPAEYDFWGQGTTVTVSSGGGGSQVQLVESGGGSVQPGGSLRLSCAASGYSYSANCVGWFRQAPGKGREGVSAINTGGETATYADFVKGRFTISRDNAKNTVYLQMNSLRAEDTAVYYCAAVGTRKYWDECSLSQHAYKNWGQGTLVTVSSGEPKSSDKTHTCPPCPAPELLGGPSVFLFPPKPKDTLMISRTPEVTCVVVDVSHEDPEVKFNWYVDGVEVHNAKTKPREEQYNSTYRVVSVLTVLHQDWLNGKEYKCKVSNKALPAPIEKTISKAKGQPREPQVCTLPPSREEMTKNQVSLSCAVKGFYPSDIAVEWESNGQPENNYKTTPPVLDSDGSFFLVSKLTVDKSRWQQGNVFSCSVMHEALHNRYTQKSLSLSPGK

SEQ ID NO: 82 - DNA, 1464 bp, synthetic construct
  source 1..1464: mol_type = other DNA
gaggtgcagctggtggaatcaggcggaggctccgtgcaggccggcggctctttgagactgtcttgtgccgtgtccggcttcaccgtgtcttctaacttcatggcctggttcagacaggctcctggcaagggcagagagtgggtcagcaccatcaccaccggcgctggaaacaccgcctacgccgactccgtgaaagggcgctttacaatcagcgaggacaactccaagaataccctgtacctgcagatgaactctctgcgggccgaggataccgccgtgtactactgtgctgctggcagaggcggcttttggcggccagctgagtacgacttctggggccaaggcaccacagtcaccgtgtcctctggcggaggtggcagccaagtgcagctggtcgaatctggaggtggctccgttcagcctggcggctctctgagactgtcttgcgccgcttccggctactcttactccgccaactgcgtgggctggttccggcaggcccccggcaaaggcagagaaggcgtgagcgccatcaacaccggcggcgaaaccgctacctatgccgatttcgtgaagggaagattcaccatctctcgggacaacgccaagaacaccgtgtatctgcagatgaactctctgagagccgaggatacagctgtgtactactgcgctgctgtgggcaccagaaagtactgggacgagtgctccctgtcccagcacgcctataagaactggggacagggcacactcgtgaccgtgtctagcggcgagcctaaaagctctgacaaaacccacacctgtcctccttgccccgctcctgagctgctgggcggcccttccgtgtttctgttccctcccaagcccaaggacacactgatgatctccagaaccccggaagtgacctgcgtggtggtggacgtgtctcacgaggaccctgaggtcaagttcaactggtacgtggatggcgtggaagtgcataatgctaagaccaagcctcgggaggaacagtacaactccacctacagagtggtttccgtgctgaccgtgctgcaccaagactggctgaacggcaaagagtacaagtgcaaggtgtccaacaaggctctgcctgcccccatcgagaagacgatctccaaggccaagggccagcctagggaacctcaggtgtgcaccctgcctccttcccgggaagagatgaccaaaaaccaggtcagcctgtcttgcgccgtgaagggcttctacccctccgacatcgccgtggaatgggagtccaacggccagcccgagaataactacaagaccacccctcctgtgctcgatagcgacggctccttcttcctggtgtctaagctgacagtggacaagtctagatggcagcagggcaacgtgttctcctgttccgtgatgcacgaggccctgcacaaccggtacacccagaagtccctgagcctgtctccaggcaag

SEQ ID NO: 83 - protein, 488 aa, synthetic construct
EVQLVESGGGSVQAGGSLRLSCAVSGFTVSSNFMAWFRQAPGKGREWVSTITTGAGNTAYADSVKGRFTISEDNSKNTAYLQMNSLRAEDTAVYYCAAGRGGFWRPAEYDFWGQGTTVTVSSGGGGSQVQLVESGGGSVQPGGSLRLSCAASGYSYSANCVGWFRQAPGKGREGVSAINTGGETATYADFVKGRFTISRDNAKNTVYLQMNSLRAEDTAVYYCAAVGTRKYWDECSLSQHAYKNWGQGTLVTVSSGEPKSSDKTHTCPPCPAPELLGGPSVFLFPPKPKDTLMISRTPEVTCVVVDVSHEDPEVKFNWYVDGVEVHNAKTKPREEQYNSTYRVVSVLTVLHQDWLNGKEYKCKVSNKALPAPIEKTISKAKGQPREPQVCTLPPSREEMTKNQVSLSCAVKGFYPSDIAVEWESNGQPENNYKTTPPVLDSDGSFFLVSKLTVDKSRWQQGNVFSCSVMHEALHNRYTQKSLSLSPGK

SEQ ID NO: 84 - DNA, 1464 bp, synthetic construct
  source 1..1464: mol_type = other DNA
gaagtgcagctggtggaatccggcggcggatctgtgcaggccgggggctccctgagactgtcttgcgccgtgtccggcttcaccgtgtcttctaacttcatggcctggtttcgccaggcacctggcaagggcagagagtgggtgtctaccatcaccaccggcgctgggaacaccgcttacgccgattctgtgaaaggccggttcaccatctccgaggataattccaagaacacagcttatctgcagatgaacagcctgagagccgaggacaccgccgtatactactgtgctgctggcagaggcggcttttggcggcctgctgagtacgacttctggggccagggcaccacagtcacagtttcctctggaggcggtggctctcaagtgcagctggtggagtctgggggaggctctgtccaacctggaggatctctgcggctgagctgcgccgcctctggctactcctacagcgccaactgcgtgggctggttcagacaggcccctggaaagggcagagaaggcgtttctgccatcaacaccggcggcgagacagccacatacgccgacttcgtgaagggcagattcaccatcagtcgggacaacgccaaaaacaccgtgtacctgcagatgaactccctccgggccgaggacaccgctgtgtactactgcgctgctgtcggcaccagaaagtactgggacgagtgctctctgagccagcacgcctacaaaaattggggccaaggcaccctcgtgacagtgagcagcggcgaacccaagtccagcgacaagacccacacctgccctccttgtcctgccccagagctgctgggcggcccttccgtgtttctgttcccacccaagcctaaggacactctgatgatcagcagaacccctgaggtgacctgtgtggtggtggacgtgtctcacgaagatcctgaagtcaagttcaactggtacgtggacggcgtggaagtgcacaacgctaagaccaagcccagagaagagcagtacaacagcacctacagagtggtctccgtgctgaccgtgctgcaccaggactggctgaacggcaaagagtataagtgcaaggtgtccaacaaggctctgcccgctcctatcgagaagaccatctccaaggccaagggccagcctcgggagcctcaggtgtgcaccctgcctccctcccgggaagagatgaccaagaaccaggtgtccttgtcttgtgctgtgaagggcttctacccttcggacatcgccgtggaatgggagtccaatggacagcccgagaacaactacaagacaacccctcctgtgctggactccgatggctccttcttcctggtgtccaagctgaccgtggataagtctaggtggcagcagggcaacgtgttctcctgctccgtgatgcacgaggccctgcataacagatacacccagaagtccctgtccctgtctcctggcaaa

SEQ ID NO: 85 - protein, 455 aa, synthetic construct
QVQLVESGGGVVQPGRSLRLSCAASGFTFSTYGMHWVRQAPGKGLEWVAVIWDDGSYKYYGDSVKGRFTISRDNSKNTLYLQMNSLRAEDTAVYYCARDGITMVRGVMKDYFDYWGQGTLVTVSSASTKGPSVFPLAPSSKSTSGGTAALGCLVKDYFPEPVTVSWNSGALTSGVHTFPAVLQSSGLYSLSSVVTVPSSSLGTQTYICNVNHKPSNTKVDKRVEPKSCDKTHTCPPCPAPELLGGPSVFLFPPKPKDTLMISRTPEVTCVVVDVSHEDPEVKFNWYVDGVEVHNAKTKPREEQYNSTYRVVSVLTVLHQDWLNGKEYKCKVSNKALPAPIEKTISKAKGQPREPQVYTLPPCREEMTKNQVSLWCLVKGFYPSDIAVEWESNGQPENNYKTTPPVLDSDGSFFLYSKLTVDKSRWQQGNVFSCSVMHEALHNHYTQKSLSLSPGK

SEQ ID NO: 86 - DNA, 1365 bp, synthetic construct
  source 1..1365: mol_type = other DNA
caggtgcagctggtggagtccggcggcggagtggtgcagccaggaagatccctgcggctgagctgtgccgcttccggcttcaccttctccacctacggcatgcactgggtgcggcaggcccccggaaagggactggagtgggtggctgtgatctgggacgacggctcctacaagtattacggcgattccgtgaagggccggttcaccatctcccgggacaactccaagaacaccctgtacctgcagatgaatagcctgagggccgaggacaccgctgtgtactactgtgcccgggacggcatcaccatggtgcggggagtgatgaaggattacttcgactactggggccagggcaccctggtgaccgtgagctccgccagtaccaaaggcccttccgtgtttcctctggccccatcctccaagagtacatctggaggcaccgctgctctgggctgcctggtgaaggactacttccccgagcccgtgaccgtcagctggaactccggcgccctgacctctggcgttcatacctttcccgccgttctgcagagctctggcctgtacagcctgtcttccgtcgtgaccgtgccttctagctctctgggaacacagacctacatctgcaacgtgaaccacaagcccagcaacaccaaggtggacaagcgggtggaacccaagtcctgcgacaaaacccacacctgtcctccttgtccagcccctgagctgctgggcggcccttctgtctttctgttccctcctaagcctaaggacacgctcatgatctcccggacacctgaagtgacctgcgtggtggtggatgtgtctcacgaggaccctgaggtgaagttcaactggtacgtggacggcgtggaagtccataacgccaagaccaagcctagagaggagcagtacaattccacctatagggtggtgagcgtgctgaccgtgctgcaccaggattggctgaatggcaaggagtacaagtgcaaggtgagcaataaggctctgcctgctcccatcgagaagaccatctccaaggctaagggccagcctagggagccccaggtgtataccctgcctccctgccgggaggagatgaccaagaaccaggtgtccctgtggtgcctggtgaagggcttctacccttccgacatcgctgtggagtgggagtccaatggccagcccgagaataattacaagaccacccctcccgtgctggattccgacggctccttcttcctgtactccaagctgaccgtggacaagagcaggtggcagcagggcaacgtgttcagctgtagcgtgatgcacgaggccctgcacaaccactacacccagaagtccctgagcctgagccccggcaag

SEQ ID NO: 87 - protein, 214 aa, synthetic construct
AIQLTQSPSSLSASVGDRVTITCRASQDISSALVWYQQKPGKAPKLLIYDASSLESGVPSRFSGSESGTDFTLTISSLQPEDFATYYCQQFNSYPLTFGGGTKVEIKRTVAAPSVFIFPPSDEQLKSGTASVVCLLNNFYPREAKVQWKVDNALQSGNSQESVTEQDSKDSTYSLSSTLTLSKADYEKHKVYACEVTHQGLSSPVTKSFNRGEC

SEQ ID NO: 88 - DNA, 642 bp, synthetic construct
  source 1..642: mol_type = other DNA
gctatccagctgacccagtcccctagctccctgagcgcctccgtgggcgacagggtgaccatcacctgcagggccagccaggatatctcctccgccctggtgtggtaccagcagaagcccggcaaggcccccaagctgctgatctatgacgctagctccctggagtccggcgtgccctccaggttcagcggctccgagtccggcaccgacttcaccctgaccatctccagcctgcagcccgaggacttcgccacctattattgtcagcagttcaatagctaccccctgaccttcggcggcggcaccaaggtggagatcaagaggaccgtggccgcccctagcgtgttcatcttccctcctagcgacgagcagctgaagagcggcaccgcctccgtggtgtgcctgctgaacaacttctatcccagggaggctaaggtgcagtggaaggtggataacgccctgcagtccggcaatagccaggagagcgtgaccgagcaggattccaaggattccacctactccctgagcagcaccctgaccctgagcaaggctgattacgagaagcacaaggtgtatgcttgtgaggtgacccaccagggcctgagcagccccgtgaccaagtccttcaacaggggcgagtgt

SEQ ID NO: 89 - protein, 16 aa, synthetic construct
GEPKSSDKTHTCPPCP

SEQ ID NO: 90 - protein, 15 aa, synthetic construct
EPKSCDKTHTCPPCP

SEQ ID NO: 91 - protein, 5 aa, synthetic construct
GGGGS

SEQ ID NO: 92 - protein, 330 aa, synthetic construct [sequence omitted]